European Patent Application EP 4 197 559 A1, published June 21, 2023. Title: immune regulatory protein-siRNA complex for anticancer activity. Applicant: KOREA INSTITUTE OF SCIENCE AND TECHNOLOGY. The sequence listing filed with the application follows.

SEQUENCE LISTING (18 sequences)

SEQ ID NO: 1 - protein, 130 aa, Artificial Sequence
  fusion protein
EEELQIIQPDKSVLVAAGETATLRCTITSLFPVGPIQWFRGAGPGRVLIYNQRQGPFPRVTTVSDTTKRNNMDFSIRIGNITPADAGTYYCIKFRKGSPDDVEFKSGAGTELSVRAKPVDGGFLGGGGCG

SEQ ID NO: 2 - DNA, 405 bp, Artificial Sequence
  The coding sequence of the fusion protein (SEQ ID NO: 1)
catatggaagaggagctgcagatcatccagcctgacaagtccgtgctggtcgctgctggtgaaactgccactctgcgttgtacgattaccagcctgttcccggtgggtccaatccagtggttccgtggtgctggtccgggtcgtgttctgatctacaaccagcgtcaaggtccgttcccgcgtgtaactaccgttagcgataccacgaagcgtaacaacatggacttttccatccgcattggcaatattaccccggccgacgcgggcacctactattgcatcaaatttcgcaaaggctccccggatgatgtagaatttaaatctggcgcaggcaccgaactgtctgttcgcgcaaaaccggtcgacggtggctttctgggtggcggtggctgcggttgaaagctt

SEQ ID NO: 3 - protein, 118 aa, Artificial Sequence
  variant SIPR alpha protein
EEELQIIQPDKSVLVAAGETATLRCTITSLFPVGPIQWFRGAGPGRVLIYNQRQGPFPRVTTVSDTTKRNNMDFSIRIGNITPADAGTYYCIKFRKGSPDDVEFKSGAGTELSVRAKP

SEQ ID NO: 4 - DNA, 354 bp, Artificial Sequence
  variant SIPR alpha protein coding sequence
gaagaggagctgcagatcatccagcctgacaagtccgtgctggtcgctgctggtgaaactgccactctgcgttgtacgattaccagcctgttcccggtgggtccaatccagtggttccgtggtgctggtccgggtcgtgttctgatctacaaccagcgtcaaggtccgttcccgcgtgtaactaccgttagcgataccacgaagcgtaacaacatggacttttccatccgcattggcaatattaccccggccgacgcgggcacctactattgcatcaaatttcgcaaaggctccccggatgatgtagaatttaaatctggcgcaggcaccgaactgtctgttcgcgcaaaaccg

SEQ ID NO: 5 - protein, 118 aa, Artificial Sequence
  wild type SIRP alpha coding sequence
EEELQVIQPDKSVLVAAGETATLRCTATSLIPVGPIQWFRGAGPGRELIYNQKEGHFPRVTTVSDLTKRNNMDFSIRIGNITPADAGTYYCVKFRKGSPDDVEFKSGAGTELSVRAKP

SEQ ID NO: 6 - DNA, 354 bp, Artificial Sequence
  wild type SIRP alpha coding sequence
gaggaggaattacaggtcattcaaccagataaatcggtcttagtagcagccggagagacagctacattgagatgtacggcgacaagccttattcccgtggggccgatccaatggtttcgcggggcaggccccggaagagaattgatttacaaccagaaggagggtcatttccctcgcgtgacgacggtcagcgacttaactaagcgtaataacatggatttttcaataagaataggcaatataactccggccgacgcagggacgtactactgtgttaaattccggaagggatctccggatgatgtcgagttcaaatctggggcgggtacagaattgagcgttcgggcaaagccc

SEQ ID NO: 7 - protein, 119 aa, Artificial Sequence
  wild type SIRPg protein
EEELQMIQPEKLLLVTVGKTATLHCTVTSLLPVGPVLWFRGVGPGRELIYNQKEGHFPRVTTVSDLTKRNNMDFSIRISSITPADVGTYYCVKFRKGSPENVEFKSGPGTEMALGAKPS

SEQ ID NO: 8 - DNA, 354 bp, Artificial Sequence
  wild type SIRPg coding sequence
gaggaagaattgcaaatgatccagccggaaaaattattactggttaccgtgggaaaaacggcgacccttcattgcacagtcacgtccctgttgccggtaggtccagttttgtggttccggggggttggaccagggcgtgaactgatctataatcaaaaggaaggtcattttccgcgcgtgaccacagtgagcgatttgactaaacggaacaatatggacttctcgatccgcatttctagtattacaccggcggacgttggcacttattattgcgtcaagttccgcaaaggaagtcctgagaacgtagagttcaagtccggtcctggcactgagatggctttgggtgctaaaccc

SEQ ID NO: 9 - protein, 118 aa, Artificial Sequence
  SIRPg variant 1 protein
EEELQIIQPEKLLLVTVGKTATLHCTITSLFPVGPVLWFRGVGPGRVLIYNQRQGPFPRVTTVSDTTKRNNMDFSIRISSITPADVGTYYCIKFRKGSPENVEFKSGPGTEMALGAKP

SEQ ID NO: 10 - DNA, 354 bp, Artificial Sequence
  SIRPg variant 1 coding sequence
gaagaggaattacaaatcatacaacctgaaaagctgttattggtcaccgtaggcaaaaccgctactctgcactgcactattacgtccctttttcctgttggtcctgtcttatggtttcgtggagtcggtccgggtcgggttcttatctataaccagcggcaaggaccattcccacgggttaccacggtttcggacacaacgaaacgcaataacatggatttttccattcggatttcaagcatcactccggccgacgttggaacttattactgcataaagtttagaaagggatctccggagaacgtagaatttaagtctggtccaggtactgagatggcccttggagcgaagccg

SEQ ID NO: 11 - protein, 118 aa, Artificial Sequence
  SIRPg variant 2 protein
EEELQIIQPEKLLLVTVGKTATLHCTVTSLFPVGPVLWFRGVGPGRVLIYNQRQGPFPRVTTVSDTTKRNNMDFSIRISSITPADVGTYYCIKFRKGSPENVEFKSGPGTEMALGAKP

SEQ ID NO: 12 - DNA, 354 bp, Artificial Sequence
  SIRPg variant 2 coding sequence
gaagaggaattacaaatcatacaacctgaaaagctgttattggtcaccgtaggcaaaaccgctactctgcactgcactgtgacgtccctttttcctgttggtcctgtcttatggtttcgtggagtcggtccgggtcgggttcttatctataaccagcggcaaggaccattcccacgggttaccacggtttcggacacaacgaaacgcaataacatggatttttccattcggatttcaagcatcactccggccgacgttggaacttattactgcataaagtttagaaagggatctccggagaacgtagaatttaagtctggtccaggtactgagatggcccttggagcgaagccg

SEQ ID NO: 13 - protein, 10 aa, Artificial Sequence
  linker peptide
GGFLGGGGCG

SEQ ID NO: 14 - DNA, 30 bp, Artificial Sequence
  linker peptide coding sequence
ggtggctttctgggtggcggtggctgcggt

SEQ ID NO: 15 - DNA, 24 bp, Artificial Sequence
  SPIR alpha_linker-F
aaacatatggaagaggagctgcag

SEQ ID NO: 16 - DNA, 27 bp, Artificial Sequence
  SPIR alpha_linker-R
aaaaagctttcaaccgcagccaccgcc

SEQ ID NO: 17 - RNA, 27 nt, Artificial Sequence
  siRNA_DNA : The 26th and 27th nucleotide  sequences are DNA
gggauauuaauacuacuucaguacaca

SEQ ID NO: 18 - RNA, 24 nt, Artificial Sequence
  siRNA ansti sense
uguacugaaguauuaauauccccg